European Patent Application EP 4 321 622 A1, published February 14, 2024. Title: A genus of Corynebacterium microorganism for producing L- arginine and a method for producing L-arginine using the same. Applicant: CJ CheilJedang Corporation. The sequence listing filed with the application follows.

SEQUENCE LISTING (20 sequences)

SEQ ID NO: 1 - protein, 513 aa, Unknown
  NCgl2608 amino acid
MSDLGPIWRWLLLVSVSICAASGLVYELALVSLSTSLNGGGIVETSLIVAGYVAALGLGALLVKPFLNWPAQTFLGVETLLGLIGGCSALVLYFTFATIGQSLWILVIATAAIGILVGAELPLLMTMIQQGRLADAKTTGSLVATLNAADYLGALLGGLAWPFVLLPWLGMMRGAAAAGMINLVAALFVGCVLLRHLLPRTHFFVSVVALLLAIAALATVLVKSDGIVATARAQLYRDPVIYSHQSDYQDIVVTERGKDRRLYLNGGLQYSTRDQHRYTESLVYPSLNPEAESVLIIGGGDGLAARELLRFPSMQITQVELDPEVIEVANTVLRSDNGGAMEDPRVSIIVDDAFTWLRSGGNNGETYDSIIIDLPDPNNDTMARLYSEEFYTLARARLNEQGRMVVQSSSAYTTPDVFWRVGATLKSAGCEQVIPYHVHVPTFGDWGFQLCGPADMELELREDTPPLTFLNDEVLVAAGVFGLDNQPRELEPSTLDHPRVVEDLRKGYRESGD

SEQ ID NO: 2 - DNA, 1542 bp, Unknown
  NCgl2608 nucleotide
atgtctgatttaggacccatctggcgctggctgttattagtttccgtctccatttgtgcggcatcggggctggtctatgagctagccctggtatccctttccaccagcttgaacggtggcggaattgtagaaacctccctcatcgtcgcaggttatgtagctgcccttggacttggtgcactgctggtcaagccgtttctcaactggcctgcacaaaccttcctcggtgtggaaaccttgctgggactcatcggtggttgctccgcgctggtgctatatttcacctttgcgaccatcggccagtccttgtggattctggtgattgccaccgctgcaattggcatcctggtcggcgctgaacttccactgctgatgaccatgatccagcaaggccgcctcgccgacgccaaaactacaggatctctggttgccaccttgaatgctgctgattaccttggcgcacttttaggtggcctggcctggccttttgtgttgctgccgtggcttggcatgatgcgcggtgccgcagcagccggaatgatcaacctcgttgcagcactattcgtgggctgtgtgctgctgcgacatttgcttccgcgcacccacttcttcgtatccgtggtggcgcttcttctcgcgatcgcagcgcttgccaccgtgttggtgaaatccgacgggatcgttgccaccgcccgcgcacagctctaccgcgaccccgtgatctattcacaccaatctgactaccaagacatcgtagtgacagaacgaggcaaagaccgacgcctctacctcaatggcggtttgcagtattccactcgtgaccagcatagatatacagaatcactggtgtatccaagccttaatccagaggcagaatcggtgttaatcatcggcggtggcgatggcctcgcagcacgggaactcctccgattcccatcaatgcagatcacccaagttgaattagacccagaagtcatcgaagtagccaacactgtgctgcgttctgacaatgggggagcgatggaagatccccgcgtgtccatcatcgtcgacgacgccttcacctggcttcgctccggcggaaacaacggcgaaacttacgattccatcatcatcgatcttcccgacccaaacaacgacaccatggccaggctgtattcagaagagttctacaccttggcccgagcacgactgaatgaacaaggccgcatggtggtgcaatcctccagcgcgtacaccaccccagatgtgttctggcgagttggagcaaccttgaaatcggcgggctgtgaacaagtcatcccatatcacgtgcatgttcccacatttggcgactggggcttccaactgtgtggccctgccgacatggaattagagcttcgggaagacaccccgccactgactttccttaatgatgaagttctggtggctgctggggtgtttgggttggataatcagcctcgtgaattggaaccttccacgctggatcatccccgcgtggtggaggatctgcgcaagggatatcgcgaatcaggcgactag

SEQ ID NO: 3 - DNA, 25 bp, Artificial Sequence
  primer 1
acctacaacaaagctctcatcaacc

SEQ ID NO: 4 - DNA, 24 bp, Artificial Sequence
  primer 2
ctaccctgtggaacacctacatct

SEQ ID NO: 5 - DNA, 34 bp, Artificial Sequence
  primer 3
tcggtacccggggatcctcggtggcggtttcggc

SEQ ID NO: 6 - DNA, 34 bp, Artificial Sequence
  primer 4
ttgcagaaagggataccagggctagctcatagac

SEQ ID NO: 7 - DNA, 34 bp, Artificial Sequence
  primer 5
ggtatccctttctgcaacgatgtgctgtgtgacg

SEQ ID NO: 8 - DNA, 34 bp, Artificial Sequence
  primer 6
tgcaggtcgactctagaaggacctggaaaagggc

SEQ ID NO: 9 - DNA, 36 bp, Artificial Sequence
  primer 7
tcggtacccggggatccagcaggccttaagggtaag

SEQ ID NO: 10 - DNA, 34 bp, Artificial Sequence
  primer 8
aggggcgctgtcttacctcggctggtgggccagc

SEQ ID NO: 11 - DNA, 36 bp, Artificial Sequence
  primer 9
ggtaagacagcgcccctagttcaaggcttgttaatc

SEQ ID NO: 12 - DNA, 37 bp, Artificial Sequence
  primer 10
tgcaggtcgactctagaaccgttgaactgcttgccag

SEQ ID NO: 13 - protein, 171 aa, Unknown
  argR amino acid
MSLGSTPSTPENLNPVTRTARQALILQILDKQKVTSQVQLSELLLDEGIDITQATLSRDLDELGARKVRPDGGRAYYAVGPVDSIAREDLRGPSEKLRRMLDELLVSTDHSGNIAMLRTPPGAAQYLASFIDRVGLKEVVGTIAGDDTVFVLARDPLTGKELGELLSGRTT

SEQ ID NO: 14 - DNA, 516 bp, Unknown
  argR nucleotide
atgtcccttggctcaaccccgtcaacaccggaaaacttaaatcccgtgactcgcactgcacgccaagctctcattttgcagattttggacaaacaaaaagtcaccagccaggtacaactgtctgaattgctgctggatgaaggcatcgatatcacccaggccaccttgtcccgagatctcgatgaactcggtgcacgcaaggttcgccccgatgggggacgcgcctactacgcggtcggcccagtagatagcatcgcccgcgaagatctccggggtccgtcggagaagctgcgccgcatgcttgatgaactgctggtttctacagatcattccggcaacatcgcgatgctgcgcaccccgccgggagctgcccagtacctggcaagtttcatcgatagggtggggctgaaagaagtcgttggcaccatcgctggcgatgacaccgttttcgttctcgcccgtgatccgctcacaggtaaagaactaggtgaattactcagcgggcgcaccacttaa

SEQ ID NO: 15 - protein, 319 aa, Unknown
  argF amino acid
MTSQPQVRHFLADDDLTPAEQAEVLTLAAKLKAAPFSERPLEGPKSVAVLFDKTSTRTRFSFDAGIAHLGGHAIVVDSGSSQMGKGETLQDTAAVLSRYVEAIVWRTYAHSNFHAMAETSTVPLVNSLSDDLHPCQILADLQTIVENLSPEEGPAGLKGKKAVYLGDGDNNMANSYMIGFATAGMDISIIAPEGFQPRAEFVERAEKRGQETGAKVVVTDSLDEVAGADVVITDTWVSMGMENDGIDRTTPFVPYQVNDEVMAKANDGAIFLHCLPAYRGKEVAASVIDGPASKVFDEAENRLHAQKALLVWLLAHQPR

SEQ ID NO: 16 - DNA, 960 bp, Unknown
  argF nucleotide
atgacttcacaaccacaggttcgccatttcctggctgatgatgatctcacccctgcagagcaggcagaggttttgaccctagccgcaaagctcaaggcagcgccgttttcggagcgtccactcgagggaccaaagtccgttgcagttctttttgataagacttcaactcgtactcgcttctccttcgacgcgggcatcgctcatttgggtggacatgccatcgtcgtggattccggcagctcacagatgggtaagggcgagaccctgcaggacaccgcagctgtattgtcccgctacgtggaagcaattgtgtggcgcacctacgcacacagcaatttccacgccatggcggagacgtccactgtgccactggtgaactccttgtccgatgatctgcacccatgccagattctggctgatctgcagaccatcgtggaaaacctcagccctgaagaaggcccagcaggccttaagggtaagaaggctgtgtacctgggcgatggcgacaacaacatggccaactcctacatgattggctttgccaccgcgggcatggatatctccatcatcgctcctgaagggttccagcctcgtgcggaattcgtggagcgcgcggaaaagcgtggccaggaaaccggcgcgaaggttgttgtcaccgacagcctcgacgaggttgccggcgccgatgttgtcatcaccgatacctgggtatccatgggtatggaaaacgacggcatcgatcgcaccacacctttcgttccctaccaggtcaacgatgaggtcatggcgaaagctaacgacggcgccatcttcctgcactgccttcctgcctaccgcggcaaagaagtggcagcctccgtgattgatggaccagcgtccaaagttttcgatgaagcagaaaaccgcctccacgctcagaaagcactgctggtgtggctgctggcccaccagccgaggtaa

SEQ ID NO: 17 - protein, 393 aa, Unknown
  carA amino acid
MSKDTTTYQGVTEIGSVPAYLVLADGRTFTGFGFGAIGTTLGEAVFTTAMTGYQETMTDPSYHRQIVVATAPQIGNTGWNDEDNESRDGKIWVAGLVIRDLAARVSNWRATTSLQQEMADQGIVGIGGIDTRALVRHLRNEGSIAAGIFSGADAQRPVEELVEIVKNQPAMTGANLSVEVSADETYVIEAEGEERHTVVAYDLGIKQNTPRRFSARGVRTVIVPAETPLEDIKQYNPSGVFISNGPGDPAAADVMVDIVREVLEADIPFFGICFGNQILGRAFGMETYKLKFGHRGINVPVKNHITGKIDITAQNHGFALKGEAGQEFETDFGTAIVTHTCLNDGVVEGVALKSGRAYSVQYHPEAAAGPNDASPLFDQFVELMDADAQKKGA

SEQ ID NO: 18 - DNA, 1182 bp, Unknown
  carA nucleotide
gtgagtaaagacaccaccacctaccagggagtcaccgagatcggatccgttccggcatacctggttcttgcagacggacgtaccttcaccggatttggctttggagctatcggcaccacccttggtgaggcagtgttcaccaccgccatgaccggttaccaagaaaccatgaccgatccttcctatcaccgccagattgttgtggctaccgcaccacagatcggtaacaccggctggaacgatgaggacaacgagtcccgcgacggcaagatttgggttgcaggccttgttatccgcgacctcgcagcacgtgtgtccaactggcgcgccaccacctccttgcagcaggaaatggcagaccaaggcatcgtcggcatcggcggaatcgacacccgcgcactggttcgccacctgcgcaacgaaggttccatcgcagcgggcatcttctccggcgctgacgcacagcgcccagttgaagaactcgtagagatcgtcaagaatcagccagcaatgaccggcgcaaacctctccgttgaggtctctgctgatgaaacctacgtcatcgaagctgagggcgaagagcgccacaccgtcgtggcctacgacctgggcattaagcaaaacaccccacgtcgtttctctgcacgcggtgttcgcaccgtcatcgtgcctgctgaaaccccattggaggacatcaagcagtacaacccatcaggcgtgtttatctccaatggccctggcgaccctgcagcagcagacgtcatggttgatatcgtccgcgaagttctggaagccgacattccattctttggcatctgcttcggcaaccagatcctcggccgcgcattcggcatggagacctacaagctgaagttcggccaccgcggcatcaacgttccagtgaagaaccacatcaccggcaagatcgacatcaccgcccagaaccacggcttcgcactcaagggtgaagcaggccaggaattcgagacagatttcggcactgcgattgtcacccacacctgccttaacgacggcgtcgttgaaggtgttgcgctgaagtccggacgcgcatactccgttcagtaccacccagaggccgctgccggcccaaatgatgcaagccccctgtttgaccagtttgttgagctgatggatgcagacgctcagaagaaaggcgcataa

SEQ ID NO: 19 - protein, 1113 aa, Unknown
  carB amino acid
MPKRSDINHVLVIGSGPIVIGQACEFDYSGTQACRVLKEEGLRVTLINSNPATIMTDPEMADHTYVEPIEPEYIDKIFAKEIEQGHPIDAVLATLGGQTALNAAIQLDRLGILEKYGVELIGADIDAIERGEDRQKFKDIVTTIGGESARSRVCHNMDEVHETVAELGLPVVVRPSFTMGGLGSGLAYNTEDLERIAGGGLAASPEANVLIEESILGWKEFELELMRDTADNVVVICSIENVDALGVHTGDSVTVAPALTLTDREFQKMRDQGIAIIREVGVDTGGCNIQFAINPVDGRIITIEMNPRVSRSSALASKATGFPIAKMAAKLAIGYTLDEITNDITGETPAAFEPTIDYVVVKAPRFAFEKFVGADDTLTTTMKSVGEVMSLGRNYIAALNKALRSLETKQQGFWTKPDEFFAGERATDKAAVLEDLKRPTEGRLYDVELAMRLGASVEELYEASSIDPWFLAELEALVQFRQKLVDAPFLNEDLLREAKFMGLSDLQIAALRPEFAGEDGVRTLRLSLGIRPVFKTVDTCAAEFEAKTPYHYSAYELDPAAESEVAPQTEREKVLILGSGPNRIGQGIEFDYSCVHAALELSRVGYETVMVNCNPETVSTDYDTADRLYFEPLTFEDVMEVYHAEAQSGTVAGVIVQLGGQTPLGLADRLKKAGVPVIGTSPEAIDMAEDRGEFGALLNREQLPAPAFGTATSFEEARTVADEISYPVLVRPSYVLGGRGMEIVYDEASLEDYINRATELSSDHPVLVDRFLDNAIEIDVDALCDGDEVYLAGVMEHIEEAGIHSGDSACALPPMTLGAQDIEKVREATKKLALGIGVQGLMNVQYALKDDILYVIEANPRASRTVPFVSKATGVNLAKAASRIAVGATIKDLQDEGMIPTEYDGGSLPLDAPIAVKEAVLPFNRFRRPDGKTLDTLLSPEMKSTGEVMGLANNFGAAYAKAEAGAFGALPTEGTVFVTVANRDKRTLILPIQRLASMGYKILATEGTAGMLRRNGIDCEVVLKASDIREGVEGKSIVDRIREGEVDLILNTPAGSAGARHDGYDIRAAAVTVGVPLITTVQGVTAAVQGIEALREGVVSVRALQELDHAVKA

SEQ ID NO: 20 - DNA, 3342 bp, Unknown
  carB nucletide
atgccaaagcgttcagatattaaccacgtcctcgtcatcggttccggccccatcgtcattggccaggcatgtgaattcgactactccggcacccaggcttgccgcgtgctgaaggaagagggactgcgcgtcaccctcatcaactccaacccagcaacgatcatgaccgacccagaaatggctgaccacacctacgtggagccaatcgagccggaatacatcgacaagattttcgctaaggagatcgagcagggccacccaatcgacgccgtcctggcaacccttggtggccagactgcacttaacgcagctatccagctggatcgcctcggcatcctggaaaagtacggcgttgaactcatcggtgcagacatcgatgccattgagcgcggcgaagatcgccagaagttcaaggatattgtcaccaccatcggtggcgaatccgcgcgttcccgcgtctgccacaacatggacgaagtccatgagactgtcgcagaacttggccttccagtagtcgtgcgtccatccttcactatgggtggcctgggctccggtcttgcatacaacaccgaagaccttgagcgcatcgcaggtggcggacttgctgcatctcctgaagcaaacgtcttgatcgaagaatccatccttggttggaaggaattcgagctcgagctcatgcgcgataccgcagacaacgttgtggttatctgctccattgaaaacgtcgacgcactgggcgtgcacaccggcgactctgtcaccgtggcacctgccctgaccctgactgaccgtgaattccagaagatgcgcgatcagggtatcgccatcatccgcgaggtcggcgtggacaccggtggatgtaacatccagttcgctatcaacccagttgatggccgcatcatcaccattgagatgaacccacgtgtgtctcgttcctccgcgctggcatccaaggcaacgggcttcccaattgccaagatggctgccaagctggctatcggatacaccctggatgagatcaccaacgacatcactggtgaaaccccagctgcgtttgagcccaccatcgactacgtcgtggtcaaggccccacgctttgctttcgagaagtttgtcggcgctgatgacactttgaccaccaccatgaagtccgtcggtgaggtcatgtccctgggccgtaactacattgcagcactgaacaaggcactgcgttccctggaaaccaagcagcagggtttctggaccaagcctgatgagttcttcgcaggggagcgcgctaccgataaggcagctgttctggaagatctcaagcgcccaaccgaaggccgcctctacgacgttgagctggcaatgcgccttggcgcaagcgtggaagaactctacgaagcatcttctattgatccttggttcctcgccgagcttgaagctctcgtgcagttccgccagaagctcgttgacgcaccattcctcaacgaagatctcctgcgcgaagcaaagttcatgggtctgtccgacctgcagatcgcagcccttcgcccagagttcgctggcgaagacggcgtacgcaccttgcgtctgtccctaggcatccgcccagtattcaagactgtggatacctgtgcagcagagtttgaagctaagactccgtaccactactccgcatacgagctggatccagcagctgagtctgaggtcgcaccacagactgagcgtgaaaaggtcctgatcttgggctccggtccaaaccgcatcggccagggcatcgagttcgactattcctgtgttcacgcagctcttgagctctcccgcgtcggctacgaaactgtcatggtcaactgcaacccagagaccgtgtccaccgactacgacaccgctgaccgcctgtacttcgagccactgaccttcgaagacgtcatggaggtctaccacgctgaggcgcagtccggcaccgtcgcaggtgttatcgtccagcttggtggccagactcctctgggcttggcagatcgtttgaagaaggctggcgtccctgtcattggtacctccccagaggcaatcgacatggctgaggaccgtggcgagttcggtgcactgctgaaccgcgagcagcttcctgctccagcattcggcaccgcaacctctttcgaagaggctcgcacagtagccgatgagatcagctacccagtgctggttcgcccttcctacgtcttgggtggccgtggcatggagattgtctacgatgaggcttccctcgaggattacatcaaccgcgcaactgagttgtcttctgaccacccagtgctggttgaccgcttcctggacaacgctattgagatcgacgtcgacgcactgtgcgacggcgacgaagtctacctggcgggcgtcatggaacacatcgaggaagccggcattcactccggtgactccgcatgtgcacttcctccaatgactttgggcgcacaggacatcgagaaggtccgcgaagcaaccaagaagctggctctgggcatcggcgtacagggcctgatgaacgtccagtacgcactcaaggacgacatcctctacgtcatcgaggcaaacccacgtgcatcccgcaccgtgccgttcgtctccaaggcaacgggcgtcaacctggccaaggcagcatcccgtatcgcagtgggcgccaccatcaaggatctccaagatgagggcatgattcctaccgagtacgacggcggctccttgccactggacgctccaatcgctgtgaaggaagcagtgttgccgttcaaccgcttccgtcgcccagatggaaagaccctggacaccctgctttccccagagatgaagtccactggcgaggtcatgggcttggccaacaacttcggcgctgcatatgcaaaggctgaagctggcgcgtttggtgcattgccaaccgaaggcaccgtcttcgtgaccgtggctaaccgcgacaagcgcaccctgatcctgccaatccagcgcctggcgtcgatgggctacaagatcctcgccaccgaaggcaccgcaggcatgctgcgccgcaacggcattgattgtgaagttgtgctcaaggcttccgacatccgcgaaggtgtagagggcaagtccatcgtggatcgtatccgcgaaggcgaagttgacctcatcctcaacaccccagctggttctgctggcgctcgccacgatggctacgatatccgcgcagcagcagtgaccgtgggtgttccactgatcaccactgtccagggtgtcaccgcagctgtccagggcattgaggccctgcgtgagggcgttgtcagcgtccgcgcgctgcaggaactcgaccacgcagtcaaggcttaa